European Patent Specification EP 3 979 830 B1, published November 26, 2025. Title: PREBIOTIC FORMULATIONS FOR PREVENTION OF NECROENTEROCOLITIS INDUCED NEURODEVELOPMENTAL DEFICIENCIES. Applicant: RESEARCH INSTITUTE AT NATIONWIDE CHILDREN'S HOSPITAL. The sequence listing filed with the application follows.

SEQUENCE LISTING (22 sequences)

SEQ ID NO: 1 - protein, 96 aa, Haemophilus influenzae
MATITKLDIIEYLSDKYHLSKQDTKNVVENFLEEIRLSLESGQDVKLSGFGNFELRDKSSRPGRNPKTGDVVPVSARRVVTFKPGQKLRARVEKTK

SEQ ID NO: 2 - protein, 136 aa, Haemophilus influenzae
MRFVTIFINHAFNSSQVRLSFAQFLRQIRKDTFKESNFLFNRRYKFMNKTDLIDAIANAAELNKKQAKAALEATLDAITASLKEGEPVQLIGFGTFKVNERAARTGRNPQTGAEIQIAASKVPAFVSGKALKDAIK

SEQ ID NO: 3 - protein, 96 aa, Haemophilus influenzae; identical to SEQ ID NO: 1

SEQ ID NO: 4 - protein, 99 aa, Escherichia coli
MALTKAEMSEYLFDKLGLSKRDAKELVELFFEEIRRALENGEQVKLSGFGNFDLRDKNQRPGRNPKTGEDIPITARRVVTFRPGQKLKSRVENASPKDE

SEQ ID NO: 5 - protein, 100 aa, Pseudomonas aeruginosa
MGALTKAEIAERLYEELGLNKREAKELVELFFEEIRQALEHNEQVKLSGFGNFDLRDKRQRPGRNPKTGEEIPITARRVVTFRPGQKLKARVEAYAGTKS

SEQ ID NO: 6 - protein, 96 aa, Haemophilus influenzae; identical to SEQ ID NO: 1

SEQ ID NO: 7 - protein, 90 aa, Escherichia coli
MNKTQLIDVIAEKAELSKTQAKAALESTLAAITESLKEGDAVQLVGFGTFKVNHRAERTGRNPQTGKEIKIAAANVPAFVSGKALKDAVK

SEQ ID NO: 8 - protein, 90 aa, Escherichia coli
MNKSQLIDKIAAGADISKAAAGRALDAIIASVTESLKEGDDVALVGFGTFAVKERAARTGRNPQTGKEITIAAAKVPSFRAGKALKDAVN

SEQ ID NO: 9 - DNA, 36 bp, Artificial Sequence
  Description of Artificial Sequence: Synthetic oligonucleotide
gcgtggcggccgccattattttcatgtagtgtattt

SEQ ID NO: 10 - DNA, 34 bp, Artificial Sequence
  Description of Artificial Sequence: Synthetic oligonucleotide
gcgtggtcgaccttttttatgtccataatctatt

SEQ ID NO: 11 - DNA, 34 bp, Artificial Sequence
  Description of Artificial Sequence: Synthetic oligonucleotide
gcgtggtcgacgaaaatatttaatatgaaaatga

SEQ ID NO: 12 - DNA, 33 bp, Artificial Sequence
  Description of Artificial Sequence: Synthetic oligonucleotide
gcgtgctcgagccaagcactatttcacgagaat

SEQ ID NO: 13 - DNA, 31 bp, Artificial Sequence
  Description of Artificial Sequence: Synthetic oligonucleotide
gcgtggtcgacgatgaaaatttgtttgattt

SEQ ID NO: 14 - DNA, 31 bp, Artificial Sequence
  Description of Artificial Sequence: Synthetic oligonucleotide
gcgtggtcgacttataaaagccagtcattag

SEQ ID NO: 15 - DNA, 34 bp, Artificial Sequence
  Description of Artificial Sequence: Synthetic oligonucleotide
gcgtgctcgagcaacaagagtatcagggtaaagc

SEQ ID NO: 16 - DNA, 34 bp, Artificial Sequence
  Description of Artificial Sequence: Synthetic oligonucleotide
gcgtggtcgactccttcccaatagatgattgatt

SEQ ID NO: 17 - DNA, 34 bp, Artificial Sequence
  Description of Artificial Sequence: Synthetic oligonucleotide
gcgtggtcgacatggtaaaacgtgaaaaaaatgt

SEQ ID NO: 18 - DNA, 31 bp, Artificial Sequence
  Description of Artificial Sequence: Synthetic oligonucleotide
gcggccgctccgccagctttttctaataact

SEQ ID NO: 19 - DNA, 34 bp, Artificial Sequence
  Description of Artificial Sequence: Synthetic primer
gcgtggctagcatgaacctgccaacaattcctaa

SEQ ID NO: 20 - DNA, 35 bp, Artificial Sequence
  Description of Artificial Sequence: Synthetic primer
gcgtggctcttccgcattaaatattttcttggttt

SEQ ID NO: 21 - DNA, 34 bp, Artificial Sequence
  Description of Artificial Sequence: Synthetic oligonucleotide
gcgtgctcgagcgcaacaaatacagtttctaata

SEQ ID NO: 22 - DNA, 34 bp, Artificial Sequence
  Description of Artificial Sequence: Synthetic oligonucleotide
gcgtggtcgacaaacctcctgataatttacaagt